European Patent Specification EP 3 782 465 B1, published August 30, 2023. Title: TRANSGENIC FISH MODEL FOR STROKE. Applicant: Universität Potsdam. The sequence listing filed with the application follows.

SEQUENCE LISTING (20 sequences)

SEQ ID NO: 1 - protein, 741 aa, Danio rerio
  protein sequence of CCM1 (KRIT1)
MMGNQELEEVFVAVIRPKNTTSLNSKEYRAKSYEILLIEVPLEGKEKKRKKVLLGTKIHADSDRTKSILEFVDETTKPISNNQGIIGKRVVHMRKFLLDGDSGGKEASLFIVPINVKDNSKSVHHPGSPSFYCLQDIMRVCSETSAHFSSSTSKMLLALDKWLAEQHTVPHAIPALFRPAPVDRVKTNVSNPAYAVEKQTDGTLHMGYTALEIKSKLMSLEKADLCIQNPLYGSDLQYTNRVDKVIINPYFGLGAPDYSKIQIPKRDKWQHSMTSVTEDKERQWVDDFPLHRSACEGDTELLSKLLDGGFSVKQLDSDHWAPIHYACWHGKVEATKLLLEKGNCNPNLLNGQLSSPLHFAAIGGHAEIVQLLLQHPEIDRHIEDQQKRSPLQVCEENKQNNWEETVNLLQQASNKPYEKVRIYRMDGSYRSVELKHGNNTTVQQIMEGMRLSQETQQYFTIWICSENLSLQLKPYHKPLQHLRMWSEIVTDLTALDPQRESPQLFLRRDVRLPLEVEKKVEDPLSILILFDEARHCLLKGFLSTSDNKLITLASLLLQIIYGNYDSKKHKQGFLNEENLKSIVPISKVKSKAHHWTNRILHEYKSLSTSEGVSKEMHHLQRLFLQNCWDIPTYGAAFFTGQVFTKASSSTHKVIRVYVGVNTKGLHLMNMETKVLHLSLEYGTFMWQLGQADQYVQIHSLENKKNFVVHTKQAGLIVKLLMKLSGQIAPNDRAVSDKYAYG

SEQ ID NO: 2 - protein, 455 aa, Danio rerio
  protein sequence of CCM2
MEEDVKKVKKPGIVSPFKRVFLKGEKGRDKKALEKSTERRALHTFSLSLPDHRIDPDILLNDYIEKEVKYLGQLTSVPGYLNPSSRTEVLQLIDNARKSHQLAGQLTSEQDAVVSLSAYNVKLVWRDGEDIILRVPIHDIAAVSYIRDDSLHLVVLKTAQEPGGSPCHSTEMSKSPTLSSLSESGAVLVEVCCLLVLAVDNKAAAEELCLLLSQVFQIVYTESTIDFLDRAIFDGATTPTRHLSIYSEDSSSKVDVKDVFEAEASTFSFQSSLEAGHSSSPSPTSAPASPQTKTASESELSTTAAELLQDYMTTLRTKLSSKEIQQFATLLHEYRNGASIHEFCINLRQLYGDSRKFLLLGLRPFIPEKDSQHFENFLETIGVKDGRGIITDSFGRYKRTTSSASDSTTNGNGAAGGSDEGTATSEGDEWDRMISDISNDIEALGSSMDQDGVPS

SEQ ID NO: 3 - protein, 210 aa, Danio rerio
  protein sequence of Pdcd10a (Ccm3a)
MTMEEMKNEADATSMVSMTLYAVMYPVFNELESVNLSAAQTLRAAFKKAEKENPGLTQDIIMKILEKKNVEINFTESLLRMAADDVEEYMIDRPEREFQDLNERARALKQILSKIPDEINDRVRFLQTIKDIASAIKELLDTVNNVFKKYQYQNRRALEHQKKEFVKHSKSFSDTLKTYFKDGKAINVFASANRLIHQTNLILQTFKTVA

SEQ ID NO: 4 - protein, 210 aa, Danio rerio
  protein sequence of Pdcd10b (Ccm3b)
MTMEEMKNEAEPNSIVSMTLYAVMYPVFNELGRINPSAAQTLRAAFVKAEKENPGLTQDIIMKILEKKNVEINFTESLLRMAADDVEEYMIKRPEQEFQDLNEKARALKHILSKIPDEINDRVRFLQTIKDIASAIKELLDTVNNVFRKYQYQNRRALEHQKKEFVKYSKSFSDTLKTYFKDGKAINVFISANRLIHQTNLILQTFKTVA

SEQ ID NO: 5 - protein, 977 aa, Danio rerio
  protein sequence of Heg1
MMETCARRVLFTAALLVLSTVIAETFSTDSDTDNPLSTETFYSRTSGLKQTSSWPGREATATAVDLSSGLGEMTEIPASVSITAAREGHSPKPLQTSTNAADWKTSMTSDETTEHLQSDTELTHNATAQWESPSSASHSITSHHPVTETRTVRDVTDLIDMDTTDSVSHTDSTYISTTNRVGERTLLSVISNSTFAYTQNSSISDAESQTSPWEEKTSGATQVNEETEETVSTVSEQTDPTFEDRNITSATLETGRSTLFQGTESQTGQPSVTGQTAKEVTDIDNPNSTPPLTVTSRDVEETDATSVSSETSYTQTSSDSASSILPFTSSERNVTSTSQESHNSTLIYSTNTGGSTEFSTGSVSSTAHEETERSSTQIVDETTLHDVTSAPPVLEDVATTIDDSLSKFPSGQSPTIPKTDDQTNTQVVPTSTHRPQVTDEATDEVSTVYSSTTTLTTTTPSVTTRQLQPHHTTVETQTQHTTIVTTDIIQVLRTTPSTAHHVPTSTTSGPQAPSTADSSDVTTLHLETSTATPGNTTAHGGRATTPFSKSSPSRTTVVVTTGHLTDKSTTETGSATTQMPLRTSASPGHVCGPKTCANGGHCVRSAEGSYYCQCLSAWTGPFCTEDVDECVNSPCPQGSVCVNTGGSFSCECDLGFDLEDGRSCTQVKTFLGTFTVNNSLHLRNLGLHELHREIQQLLNASLSIFHGYRRFTLGKRDGQGVQIPVVSMFSLSSNVTSADVFNSIQMSLNNCSRTYSHCPIKLQHQLSYHVESLCMAQKTKCDVQYSDCSDISGIPNCQCLPGYFKRNPEDMTCRDCGDGLKLVNGKCVECMFGFGGFNCNNFYKLIAVVVSPAGGALLLIVVIALIVTCCKKDKNDINKIIFKSGELQMSPYAEFPKSNRVSMEWGRETIEMQENGSTKNLLQMTDIYYSPALRNSDLERNGLYPFSGLPGSRHSCIYPAQWNPSFLSDDSRRRDYF

SEQ ID NO: 6 - DNA, 2226 bp, Danio rerio
  Coding nucleotide sequence of ccm1 (krit1)
atgatgggaaaccaagagctagaggaggtgtttgttgctgttatccgaccaaaaaacacaaccagcctcaactccaaagaataccgtgctaaatcctatgagattttacttatcgaagttcccctggagggaaaagagaaaaagcggaagaaagtgctgcttgggactaaaatccacgccgacagtgaccggacaaagtcaattctggagtttgtggatgaaaccaccaagcccatatccaataaccagggcataatagggaagcgtgtcgtgcacatgaggaagttcctgttagatggagacagtggaggaaaagaggcctcgttatttattgtgccaattaatgtcaaagacaacagcaagtccgtgcatcaccctgggagccccagtttctactgccttcaggacatcatgcgtgtgtgtagtgaaaccagtgctcatttctcctccagcacctcaaagatgctgctcgctctcgacaagtggttagcggagcagcacactgtgcctcacgctattcctgctctgttccggccggctccggtggaccgtgtgaaaactaacgtgagtaacccggcgtacgcagtggagaagcagacagacgggacgctgcacatgggctacacggctctggagatcaagagtaaactgatgtctctggagaaagcagatctgtgcatccagaacccgctgtacggctcagatctgcagtacaccaacagagtggacaaagtcatcatcaacccttactttggcttgggagctccagattactccaaaatccagattccaaagagagacaaatggcagcacagcatgaccagcgtcaccgaagacaaagagcgccagtgggtggatgatttccctctgcaccgaagcgcctgtgagggagacactgagcttttgtctaaattgctggatggcggattctcagtcaaacagctggacagcgaccattgggcacccattcattatgcatgctggcatgggaaggtggaggccactaaactgctgctggagaaaggcaactgtaaccccaacctgctgaacggccagctgagctctcctttacacttcgcagctatcggcggtcatgcagaaatcgtgcagctcctcctgcagcacccagagatcgacagacacatcgaggaccagcagaaacgatcgccgcttcaagtatgtgaagaaaacaagcagaacaactgggaggaaaccgtgaatctccttcaacaagccagcaataaaccatacgagaaggtgaggatttaccgtatggatggatcgtaccgctctgtggagctgaagcatgggaacaacaccaccgtgcagcagatcatggagggcatgagattatcacaggagacccagcagtattttaccatctggatctgctccgaaaaccttagtctgcagctgaagccgtaccacaagcccttgcagcacttacggatgtggagcgagatcgtgacggatctcactgctctggatccacagagagaaagtccacagctcttcctgcgcagagacgttcggctgcctttagaggtcgagaaaaaggttgaagatccgctgtccatcctcatcctatttgatgaagctcgtcactgcctccttaaaggtttcctctcgacgtcagataacaagctaatcacgctcgcaagcctcctcctgcagatcatctacggaaactacgacagcaagaagcacaaacagggctttctaaatgaggaaaacctgaaatccatagttcccatttcaaaggtcaagagcaaagcacatcactggactaacaggatacttcacgagtacaagagtctgagcactagtgagggtgtgagtaaagaaatgcatcacctccagaggctcttcctgcagaactgctgggatattcctacttatggtgcagcgtttttcacaggacaggtcttcactaaagccagctccagcacacacaaggtgatccgcgtgtatgtgggcgtcaacaccaaaggcctgcatctgatgaacatggagacaaaagtgcttcacctcagtctggagtatgggacatttatgtggcagctgggtcaggctgatcaatacgtgcaaatccacagtctggagaacaagaagaactttgtcgttcacaccaaacaggctggtcttatcgtgaagctgctgatgaagctgagtggacaaattgcaccaaacgacagagctgtgtctgataaatatgcgtatgggtaa

SEQ ID NO: 7 - DNA, 1368 bp, Danio rerio
  Coding nucleotide sequence of ccm2
atggaggaggatgtaaagaaagtcaaaaagccaggtatcgtgtctccgttcaagcgggtgtttctgaaaggggagaagggtagggataagaaggctctggagaagtccactgaacgcagggccctccacaccttctctctctctctcccagaccaccgtatcgacccagatattctgctcaatgactacatcgagaaggaagttaagtatctgggacagctgacctcagttcctggatacctgaatccctccagccgcactgaagttctgcagctcattgacaatgccaggaagtctcatcagttggctgggcagctgacctcagagcaggatgctgttgtcagtttatcagcgtacaatgtgaagcttgtgtggcgtgatggagaggacatcattctgcgcgtacccatccacgacattgcagctgtgtcctacatcagagacgactcgcttcatctagtggtgctaaaaacagctcaggagcccggaggttccccatgtcatagtacagagatgtcgaaatctcccactctgagctctctatctgagagtggggctgtgctggtggaggtctgctgtctgcttgtgctggctgttgacaacaaggctgcagcagaggagctctgtcttctactcagtcaagtcttccagatcgtctataccgagtccaccatcgacttcctagacagggccatctttgatggagccacaacacccaccaggcatctctcaatctatagtgaagactcctcaagtaaagttgatgtcaaagatgtgtttgaggccgaggcaagcacattctcgttccagagttctctagaggcgggacattcctctagcccctcccccacctcggccccggcctcgccacaaaccaaaacagccagtgagagcgaactgagcacaacagctgctgaactgctgcaagactacatgaccacattgaggacaaagctttcgtccaaagagatccagcagtttgccacactgttacatgaatacagaaacggcgcctccatccatgagttctgtatcaacctgcggcagctttatggagacagcaggaagttccttctcctcggactgcggccgttcatccccgagaaggacagccagcattttgagaactttctggagaccatcggcgtgaaggatggccgcggaatcatcacagacagtttcggccgttataagcgcacgacgagctctgcgtctgactccaccacgaacggaaacggtgctgcgggcggatcagatgagggaacagccacctctgagggcgacgaatgggaccgcatgatttcagacataagcaatgacattgaagccttaggaagcagcatggatcaagacggcgtgccatcttga

SEQ ID NO: 8 - DNA, 633 bp, Danio rerio
  Coding nucleotide sequence of pdcd10a (ccm3a)
atgacaatggaagagatgaagaatgaagcggacgcgacctccatggtatccatgaccctctacgccgtgatgtacccggtgttcaatgagctggagagtgtaaatctgtctgcggcacagactctgcgagctgctttcaaaaaggcagagaaggaaaacccaggactgactcaggacattatcatgaaaatactggagaagaagaacgtggagatcaacttcaccgagtctttattacgcatggctgctgatgatgttgaggagtacatgattgacaggcccgagcgggagttccaggacctgaatgaaagagctcgcgcgctgaaacagatcctcagcaaaatcccagacgaaattaatgaccgagtccgattcctgcagacaatcaaagatatagccagtgccataaaagagctgctggacacagtgaacaacgtcttcaagaaatatcagtaccagaacagaagggcacttgagcatcagaagaaagagtttgtgaaacattcgaaaagcttcagcgacactctgaaaacatacttcaaagacggaaaggcaataaacgtgtttgccagtgccaaccggctcatccaccaaaccaacttgatactgcagaccttcaaaactgtcgcatag

SEQ ID NO: 9 - DNA, 633 bp, Danio rerio
  Coding nucleotide sequence of pdcd10b (ccm3b)
atgacaatggaagagatgaagaatgaagctgagccaaattcaatagtctctatgacattgtacgcagtcatgtatccagtcttcaatgagttggggaggataaacccgtcagcagcacagacattgcgggcagcatttgtcaaagcagagaaggagaacccagggctcactcaagatatcattatgaagatactggagaagaagaatgtggagatcaacttcacagagtcactactgcgcatggctgcagatgatgtggaggagtacatgattaagagacctgaacaggagttccaggacctgaatgagaaagcacgagctctaaaacatatcctgagtaaaatcccagatgagatcaacgacagagtgcgcttcctacagactatcaaagacatcgccagtgctataaaggagctgctggacacagtcaacaatgtttttaggaagtatcagtaccagaatcgcagggcacttgaacaccaaaagaaggagtttgtgaagtactccaaaagcttcagtgatacgctgaaaacatacttcaaagacggaaaggcaataaacgtctttatcagtgccaacaggcttatccaccaaactaacttgatactgcagaccttcaaaaccgtcgcctag

SEQ ID NO: 10 - DNA, 2934 bp, Danio rerio
  Coding nucleotide sequence of heg1
atgatggaaacgtgcgctcgccgtgtgcttttcacggccgctctgctcgtcctcagtactgtgatagcggaaactttctccacagactcggacaccgataatccactgagtacagaaactttttatagccgaacaagtggcttgaaacaaacctcctcctggccagggagagaggccactgccacagccgtggatctatcgagcggactgggagagatgacggagattcccgccagtgtatccatcactgcagcccgagagggacattcaccaaaacctttacaaacctctacaaatgcagcggattggaagaccagtatgacctcagatgagacaacagaacatcttcaatctgacactgagcttacccataatgcgaccgcccaatgggagagtccatcatcagcatctcacagcattaccagccaccatccagtaacagagacacgaaccgtgcgagatgtaacagatctgatagacatggacaccacagactcagtctcccacactgatagcacctacatttccacaaccaaccgagttggagaacgcacactgctctcagtgatctccaacagcacctttgcgtacacccagaactcaagcatctctgatgcagagtctcaaacgtccccatgggaggagaagacatcaggagccacccaagtcaatgaggaaactgaagaaactgtgtcaacagtgtccgaacagactgatcccacttttgaagaccgcaatatcaccagtgcaactctggagactgggcggtcaacattattccaaggcactgagtcacagacaggacaacctagtgtcacaggacagaccgctaaggaggtgactgatatcgacaatccaaattcaacaccgcctctcacagtaaccagtagggatgttgaggaaacagatgccacatcagtgagcagtgagacatcttatacacaaaccagcagtgactctgcctcctcaatcttgccttttacttctagtgaacgcaatgtcactagcacgtcccaagagagccataattccacactcatttattccacaaatactggtggttccactgagttttcgactggatcagtgagctctaccgcccatgaagaaactgaacggtcttcaactcaaatagtagatgagacaacccttcatgatgttacttctgcacccccagtgcttgaagatgtagccacaactatcgatgactcgctttccaagttcccttccggccaatcgcctaccatccctaaaaccgatgaccaaaccaacacacaagtggtgccaacatcaactcataggccacaggttacagatgaagccaccgatgaggtgtctacagtttacagttctaccactactttaactaccacaactccttctgtcaccactagacaactccaaccacaccacaccacagtggaaacccaaacacaacacactaccattgttaccaccgatatcattcaggtactgcgaacgacaccttctacagcccatcatgtgcctacatcgactaccagtggaccacaggctccaagtacagctgattcttctgacgtcaccacattgcacttggaaaccagcacagccacgccggggaacactacggcgcacggtggacgtgcaacaacgccttttagcaagagcagcccgagtagaacaactgtggtagtgaccactggacatctcactgacaaaagcactacagagacaggaagcgcaaccacgcagatgcctcttagaacatcagcatcaccaggtcatgtatgtggacctaaaacctgtgcaaatggaggtcattgtgttagatcagctgaaggaagttactactgtcagtgtctctccgcatggaccggacccttctgcactgaagatgtggacgagtgtgtgaacagtccatgtcctcagggttcagtgtgtgtcaacacaggtggttctttcagctgtgaatgtgacctgggctttgacctggaggatggccgcagttgtacacaagtcaagacatttttgggcactttcacagtcaacaactctcttcatctcagaaatttaggtctgcacgagctacacagagagatccaacagctgctcaatgcttctctctccatcttccatggttatagacgctttaccctgggtaaaagagatggacaaggtgtgcaaatcccagtggtgagcatgttttcactctcctccaatgtgaccagcgcggatgttttcaacagcatccagatgtcccttaacaactgcagccggacatactcgcactgtcccattaaacttcagcaccagctctcctatcacgtggagagcctgtgcatggcccagaagaccaagtgtgatgtgcagtactcagattgctcggatattagcgggattcccaactgtcagtgccttcctgggtactttaaaaggaacccagaagacatgacctgcagagactgtggagatggactcaagcttgttaatggcaaatgtgtcgaatgcatgtttggatttggaggtttcaactgcaataatttctataagctgatagccgtggtggtctcgcctgctggaggagctcttctgttgattgtggtcattgctcttattgtcacctgctgcaaaaaagacaaaaacgacatcaacaagatcatcttcaaaagtggagagcttcagatgtcgccatacgcagagtttcctaagagcaatcgcgtgtccatggagtggggtagagagactatcgagatgcaggagaacggcagtacaaaaaacctcctgcaaatgactgacatttattactcgcctgcactgagaaactccgacctggagcgtaatggtctgtatccattctcgggccttcctggttcaaggcattcctgcatctatccggctcagtggaacccttccttcttaagcgacgattcacgccgaagagactacttttga

SEQ ID NO: 11 - DNA, 11311 bp, Artificial Sequence
  Plasmid Sequenz of pDestTol2_UAS:mCherry-Krit1,alpha-cry:EGFP
taccacctaaattgtaagcgttaatattttgttaaaattcgcgttaaatttttgttaaatcagctcattttttaaccaataggccgaaatcggcaaaatcccttataaatcaaaagaatagaccgagatagggttgagtgttgttccagtttggaacaagagtccactattaaagaacgtggactccaacgtcaaagggcgaaaaaccgtctatcagggcgatggcccactacgtgaaccatcaccctaatcaagttttttggggtcgaggtgccgtaaagcactaaatcggaaccctaaagggagcccccgatttagagcttgacggggaaagccggcgaacgtggcgagaaaggaagggaagaaagcgaaaggagcgggcgctagggcgctggcaagtgtagcggtcacgctgcgcgtaaccaccacacccgccgcgcttaatgcgccgctacagggcgcgtcccattcgccattcaggctgcgcaactgttgggaagggcgatcggtgcgggcctcttcgctattacgccagctggcgaaagggggatgtgctgcaaggcgattaagttgggtaacgccagggttttcccagtcacgacgttgtaaaacgacggccagtgagcgcgcgtaatacgactcactatagggcgaattgggtaccaaatagtaggaattacccacctgtacaagtgctgaaaacttggatgaataagcccgtttgccattttctactgctattttaaatcttttctgtatttgtctgcatttgtctttacccttgaataaatgttttagttgttttttttcaattatgactgtgtttaacagacattattacaataatatgtaatagtagtacacactattattatgtaatagtacttgttgactgtatttgagaactggaccgagtgagtgttacgtcacccattcaaaatgacttacttctggctccaacaaaatgaagttaattcagttgccatttttcactgtatggacatcgccgtgttggagctagacgtcgccaataagcaagaaagagccgagatgcgtcgagtctgagtcaccgttcctatggcaacccctctaaccaatcagaagtaagcttgttggaagtccacagcctaccacttgaaagcgggctgcacaaaatctgtcaaacgttttgaacgttggatgtgagagcacatacttttattaaggcatctggttggtcagtttataatatcaacaacttgggctacagaaaagaaaagttattacagaaattatgattaacaagtacatgttaaataaagattttaatatgaatgccaccactggagcattcatgccatttggagcttcttcctgtttggatcactagaaggaggaggtcactcattacagttctcatatacagtcgttggttggttggttggttggttggttggtagattgattgattgattgattgattgattgattgattgattgattgattgattgattgattgattgattgattgattgattgattgattgattgattgattgattggtagtcaaaataagaaataatttccacagattcattacagaaatgattaaatgcatacataaaaaactggggggggggggatacaacaacacacttaagtcacatttgcctacgtaaagaaaagtaaagaaaatcaatagctatattttacatctcctttttttgctgtcttttaattagccttgttttgctgttatcttgattgaaactgtaacttcttcacctgcttcttttctttgtaggttttgccagcccagaaacaggcatggctgtgcaaggccagagcaccatgcacaatgcgctgcatgtcttcatgaacggctcaatgtcctcagtccagggctcagccaacgaccccatcttcctccttcaccatgctttcattgacaggtaacaaacacgtcatgacattagactgcacagtttttgacaaagttcatacaatctgttgtttatagctgctacaattagtgaagtttgtgaatgtacttggatgagcagcgaaagatcaattgagatcaattgttagagtttggttgccctgcagagcaaagaacaaaaaataatctggtggctttactgcgtgaggttattattggtggaatagaaacacaaaacataattgcatttatttgtttaattttttatcttatcttaactttcatcttgcatatttgtttcttacatcatttctagcatctttgagcgctggctaagaactcatcagcctccccggtccatctacccacgtaccaatgcaccaattggccacaatgacggctactacatggtgccattccttcctctttataggaatggagactacctcctgtccaacaaggctcttggatacgagtacgcctacctgttggacccaggtcattgcacaacaccagaaatgccctctgatctgcaaaagacgtgaatatctgttcagacacccatatccactctgttccacacaggtcagaggtttgtccaggagttcttgacagaggtgtaaaaagtactcaaaaattttactcaagtgaaagtacaagtacttagggaaaattttactcaattaaaagtaaaagtatctggctagaatcttacttgagtaaaagtaaaaaagtactccattaaaattgtacttgagtattaaggaagtaaaagtaaaagcaagaaagaaaactagagattcttgtttaagcttttaatctcaaaaaacattaaatgaaatgcatacaaggttttatcctgctttagaactgtttgtatttaattatcaaactataagacagacaatctaatgccagtacacgctactcaaagttgtaaaacctcagatttaacttcagtagaagctgattctcaaaattgttagtgtcaagcctagctcttttggggctgaaaagcaatcctgcagtgctgaaaagcctctcacaggcagccgatgcgggaagaggtgtattagtcttgatagagaggctgcaaatagcaggaaacgtgagcagagactccctggtgtctgaaacacaggccagatgggccctcgagcaggaaacagctatgaccatgattacgccaagctatcaactttgtatagaaaagttggtaatacgactcactatagggcgaattgggtaccgggccccccctcgaggtcgacggtatcgataagcttaggcctccaaggcggagtactgtcctccgggctggcggagtactgtcctccggcaaggtcggagtactgtcctccgacactagaggtcggagtactgtcctccgacgcaaggcggagtactgtcctccgggctggcggagtactgtcctccggcaaggtcggagtactgtcctccgacactagaggtcggagtactgtcctccgacgcaaggcggagtactgtcctccgggctggcggagtactgtcctccggcaagggtcgactctagagggtatataatggatcccatcgcgtctcagcctcactttgagctcctccacacgaattcctgcagcccgggggatccactagttctagagcggccgccaccgcggtggagctccagcttttgttccctttagtgagggttaattcaagtttgtacaaaaaagcaggctcatggcatggtgagcaagggcgaggacgacaacatggccatcatcaaggagttcatgcgcttcaaggtgcacatggagggctccgtgaacggccacgagttcgagatcgagggcgagggcgagggccgcccctacgagggcacccagaccgccaagctgaaggtgaccaagggcggccccctgcccttcgcctgggacatcctgtcccctcagttcatgtacggctccaaggcctacgtgaagcaccccgccgacatccccgactacttgaagctgtccttccccgagggcttcaagtgggagcgcgtgatgaacttcgaggacggcggcgtggtgaccgtgacccaggactcctccctgcaggacggcgagttcatctacaaggtgaagctgcgcggcaccaacttcccctccgacggccccgtaatgcagaagaagaccatgggctgggaggcctcctccgagcggatgtaccccgaggacggcgccctgaagggcgagatcaagcagaggctgaagctgaaggacggcggccactacgacgccgaggtcaagaccacctacaaggccaagaagcccgtgcagctgcccggcgcctacaacgtcaacatcaagctggacatcacctcccacaacgaggactacaccatcgtggaacagtacgagcgcgccgagggccgccactccaccggcggcatggacgagctgtacaagggaggcgctgcaggaggctctagaatgggaaaccaagagctagaggaggtgtttgttgctgttatccgaccaaaaaacacaaccagcctcaactccaaagaataccgtgctaaatcctatgagattttacttatcgaagttcccctggagggaaaagagaaaaagcggaagaaagtgctgcttgggactaaaattcacgccgacagtgaccggacaaagtcaattctggagtttgtggatgaaaccaccaagcccatatccaataaccagggcataatagggaagcgtgttgtgcacatgaggaagttcctgttagatggagacagtggaggaaaagaggcctcgttatttattgtgccaattaatgtcaaagacaacagcaagtccgtgcatcaccctgggagccccagtttctactgccttcaggacatcatgcgtgtgtgtagtgaaaccagtgctcatttctcctccagcacctcaaagatgctgctcgctctcgacaagtggttagcggagcagcacactgtgcctcacgctattcctgctctgttccggccggctccggtggaccgtgtgaaaactaacgtgagtaacccggcgtacgcagtggagaagcagacagacgggacgctgcacatgggctacacggctctggagatcaagagtaaactgatgtctctggagaaagcagatctgtgcatccagaacccgctgtacggctcagatctgcagtacaccaacagagtggacaaagtcatcatcaacccttactttggcttgggagctccagattactccaaaatccagattccaaagagagacaaatggcagcacagcatgaccagcgtcaccgaagacaaagagcgccagtgggtggatgatttccctctgcaccgaagcgcctgtgagggagacactgagcttttgtctaaattgctggatggcggattctcagtcaaacagctggacagcgaccattgggcacccattcattatgcatgctggcatgggaaggtggaggccactaaactgctgctggagaaaggcaactgtaaccccaacctgctgaacggccagctgagctctcctttacacttcgcagctatcggcggtcatgcagaaatcgtgcagctcctcctgcagcacccagagatcgacagacacatcgaggaccagcagaaacgatcgccgcttcaagtatgtgaagaaaacaagcagaacaactgggaggaaaccgtgaatctccttcaacaagccagcaataaaccatacgagaaggtgaggatttaccgtatggatggatcgtaccgctctgtggagctgaagcatgggaacaacaccaccgtgcagcagatcatggagggcatgagattatcacaggagacccagcagtattttaccatctggatctgctccgaaaaccttagtctgcagctgaagccgtaccacaagcccttgcagcacttacggatgtggagcgagatcgtgacggatctcactgctctggatccacagagagaaagtccacagctcttcctgcgcagagacgttcggctgcctttagaggtcgagaaaaaggttgaagatccgctgtccatcctcatcctatttgatgaagctcgtcactgcctccttaaaggtttcctctcgacgtcagataacaagctaatcacgctcgcaagcctcctcctgcagatcatctacggaaactacgacagcaagaagcacaaacagggctttctaaatgaggaaaacctgaaatccatagttcccatttcaaaggtcaagagcaaagcacatcactggactaacaggatacttcacgagtacaagagtctgagcactagtgagggtgtgagtaaagaaatgcatcacctccagaggctcttcctgcagaactgctgggatattcctacttatggtgcagcgtttttcacaggacaggtcttcactaaagccagctccagcacacacaaggtgatccgcgtgtatgtgggcgtcaacaccaaaggcctgcatctgatgaacatggagacaaaagtgcttcacctcagtctggagtatgggacatttatgtggcagctgggtcaggctgatcaatacgtgcaaatccacagtctggagaacaagaagaactttgtcgttcacaccaaacaggctggtcttatcgtgaagctgctgatgaagctgagtggacaaattgcaccaaacgacagagctgtgtctgataaatatgcgtatgggtaaacccagctttcttgtacaaagtggaattcactagtgatttaatagtgtgcattcagtgcaggatgttatgtatttattttctgtagtgcaaactttttcaaagaattttccagtctaagcttttcagtcaagaaaaaaaaaggcgtctgattatctgtgatattttaaataattagctcttaaatctggtgaaccaagtggccacaacacattaaatactgacgttctacagccatgtagcttcatctggtctggtttgttttggcaggcacttattttccggtgatagttggccacaagagtattgtctgagccattcagtgctagactgtcattctcaggtcagaatccaccccactgattctgctgacaacactgttcccaccatgagataatgccattccagagagatccatttgtaagcccctctttctgcagcacaggtatataaccagggctctgcctccactaaggccggcacacatcatttggggatctttgtactgtactagcctctattagcctcctacttgcgttcagttcacatcttttgttcatcaggtgcaataagttacagtaaggagttaccaggtctgacattaatcgaattccaccatggtgagcaagggcgaggagctgttcaccggggtggtgcccatcctggtcgagctggacggcgacgtaaacggccacaagttcagcgtgtccggcgagggcgagggcgatgccacctacggcaagctgaccctgaagttcatctgcaccaccggcaagctgcccgtgccctggcccaccctcgtgaccaccctgacctacggcgtgcagtgcttcagccgctaccccgaccacatgaagcagcacgacttcttcaagtccgccatgcccgaaggctacgtccaggagcgcaccatcttcttcaaggacgacggcaactacaagacccgcgccgaggtgaagttcgagggcgacaccctggtgaaccgcatcgagctgaagggcatcgacttcaaggaggacggcaacatcctggggcacaagctggagtacaactacaacagccacaacgtctatatcatggccgacaagcagaagaacggcatcaaggtgaacttcaagatccgccacaacatcgaggacggcagcgtgcagctcgccgaccactaccagcagaacacccccatcggcgacggccccgtgctgctgcccgacaaccactacctgagcacccagtccgccctgagcaaagaccccaacgagaagcgcgatcacatggtcctgctggagttcgtgaccgccgccgggatcactctcggcatggacgagctgtacaagggcggtggaagatctgggaattcaaggcctctcgagcctctagattctgcagccctatagtgagtcgtattacgtagatccagacatgataagatacattgatgagtttggacaaaccacaactagaatgcagtgaaaaaaatgctttatttgtgaaatttgtgatgctattgctttatttgtaaccattataagctgcaataaacaagttaacaacaacaattgcattcattttatgtttcaggttcagggggaggtgtgggaggttttttccaactttattatacatagttgataattcactggccgtcgttttacatcgatgatgatccagacatgataagatacattgatgagtttggacaaaccacaactagaatgcagtgaaaaaaatgctttatttgtgaaatttgtgatgctattgctttatttgtaaccattataagctgcaataaacaagttaacaacaacaattgcattcattttatgtttcaggttcagggggaggtgtgggaggttttttaaagcaagtaaaacctctacaaatgtggtatggctgattatgatcctctagatcagatctgcgaagatacggccacgggtgctcttgatcctgtggctgattttggactgtgctgctcgcagctgctgatgaatcacatacttcctccattttcttccactgattgactgttataatttccctaatttccaggtcaaggtgctgtgcattgtggtaatagatgtgacatgacgtcacttccaaaggaccaatgaacatgtctgaccaatttcatataatgtgaaaacgattttcataggcagaataaataacatttaaattaaactgggcatcagcgcaattcaattggtttggtaatagcaagggaaaatagaatgaagtgatctccaaaaaataagtactttttgactgtaaataaaattgtaaggagtaaaaagtacttttttttctaaaaaaatgtaattaagtaaaagtaaaagtattgatttttaattgtactcaagtaaagtaaaaatccccaaaaataatacttaagtacagtaatcaagtaaaattactcaagtactttacacctctggttcttgaccccctaccttcagcaagcccagcagatccactagttctagagcggccgccaccgcggtggagctccagcttttgttccctttagtgagggttaattgcgcgcttggcgtaatcatggtcatagctgtttcctgtgtgaaattgttatccgctcacaattccacacaacatacgagccggaagcataaagtgtaaagcctggggtgcctaatgagtgagctaactcacattaattgcgttgcgctcactgcccgctttccagtcgggaaacctgtcgtgccagctgcattaatgaatcggccaacgcgcggggagaggcggtttgcgtattgggcgctcttccgcttcctcgctcactgactcgctgcgctcggtcgttcggctgcggcgagcggtatcagctcactcaaaggcggtaatacggttatccacagaatcaggggataacgcaggaaagaacatgtgagcaaaaggccagcaaaaggccaggaaccgtaaaaaggccgcgttgctggcgtttttccataggctccgcccccctgacgagcatcacaaaaatcgacgctcaagtcagaggtggcgaaacccgacaggactataaagataccaggcgtttccccctggaagctccctcgtgcgctctcctgttccgaccctgccgcttaccggatacctgtccgcctttctcccttcgggaagcgtggcgctttctcatagctcacgctgtaggtatctcagttcggtgtaggtcgttcgctccaagctgggctgtgtgcacgaaccccccgttcagcccgaccgctgcgccttatccggtaactatcgtcttgagtccaacccggtaagacacgacttatcgccactggcagcagccactggtaacaggattagcagagcgaggtatgtaggcggtgctacagagttcttgaagtggtggcctaactacggctacactagaaggacagtatttggtatctgcgctctgctgaagccagttaccttcggaaaaagagttggtagctcttgatccggcaaacaaaccaccgctggtagcggtggtttttttgtttgcaagcagcagattacgcgcagaaaaaaaggatctcaagaagatcctttgatcttttctacggggtctgacgctcagtggaacgaaaactcacgttaagggattttggtcatgagattatcaaaaaggatcttcacctagatccttttaaattaaaaatgaagttttaaatcaatctaaagtatatatgagtaaacttggtctgacagttaccaatgcttaatcagtgaggcacctatctcagcgatctgtctatttcgttcatccatagttgcctgactccccgtcgtgtagataactacgatacgggagggcttaccatctggccccagtgctgcaatgataccgcgagacccacgctcaccggctccagatttatcagcaataaaccagccagccggaagggccgagcgcagaagtggtcctgcaactttatccgcctccatccagtctattaattgttgccgggaagctagagtaagtagttcgccagttaatagtttgcgcaacgttgttgccattgctacaggcatcgtggtgtcacgctcgtcgtttggtatggcttcattcagctccggttcccaacgatcaaggcgagttacatgatcccccatgttgtgcaaaaaagcggttagctccttcggtcctccgatcgttgtcagaagtaagttggccgcagtgttatcactcatggttatggcagcactgcataattctcttactgtcatgccatccgtaagatgcttttctgtgactggtgagtactcaaccaagtcattctgagaatagtgtatgcggcgaccgagttgctcttgcccggcgtcaatacgggataataccgcgccacatagcagaactttaaaagtgctcatcattggaaaacgttcttcggggcgaaaactctcaaggatcttaccgctgttgagatccagttcgatgtaacccactcgtgcacccaactgatcttcagcatcttttactttcaccagcgtttctgggtgagcaaaaacaggaaggcaaaatgccgcaaaaaagggaataagggcgacacggaaatgttgaatactcatactcttcctttttcaatattattgaagcatttatcagggttattgtctcatgagcggatacatatttgaatgtatttagaaaaataaacaaataggggttccgcgcacatttccccgaaaagtg

SEQ ID NO: 12 - DNA, 11314 bp, Artificial Sequence
  Plasmid Sequenz of pDestTol2_UAS:EGFP-Krit1,alpha-cry:EGFP
taccacctaaattgtaagcgttaatattttgttaaaattcgcgttaaatttttgttaaatcagctcattttttaaccaataggccgaaatcggcaaaatcccttataaatcaaaagaatagaccgagatagggttgagtgttgttccagtttggaacaagagtccactattaaagaacgtggactccaacgtcaaagggcgaaaaaccgtctatcagggcgatggcccactacgtgaaccatcaccctaatcaagttttttggggtcgaggtgccgtaaagcactaaatcggaaccctaaagggagcccccgatttagagcttgacggggaaagccggcgaacgtggcgagaaaggaagggaagaaagcgaaaggagcgggcgctagggcgctggcaagtgtagcggtcacgctgcgcgtaaccaccacacccgccgcgcttaatgcgccgctacagggcgcgtcccattcgccattcaggctgcgcaactgttgggaagggcgatcggtgcgggcctcttcgctattacgccagctggcgaaagggggatgtgctgcaaggcgattaagttgggtaacgccagggttttcccagtcacgacgttgtaaaacgacggccagtgagcgcgcgtaatacgactcactatagggcgaattgggtaccaaatagtaggaattacccacctgtacaagtgctgaaaacttggatgaataagcccgtttgccattttctactgctattttaaatcttttctgtatttgtctgcatttgtctttacccttgaataaatgttttagttgttttttttcaattatgactgtgtttaacagacattattacaataatatgtaatagtagtacacactattattatgtaatagtacttgttgactgtatttgagaactggaccgagtgagtgttacgtcacccattcaaaatgacttacttctggctccaacaaaatgaagttaattcagttgccatttttcactgtatggacatcgccgtgttggagctagacgtcgccaataagcaagaaagagccgagatgcgtcgagtctgagtcaccgttcctatggcaacccctctaaccaatcagaagtaagcttgttggaagtccacagcctaccacttgaaagcgggctgcacaaaatctgtcaaacgttttgaacgttggatgtgagagcacatacttttattaaggcatctggttggtcagtttataatatcaacaacttgggctacagaaaagaaaagttattacagaaattatgattaacaagtacatgttaaataaagattttaatatgaatgccaccactggagcattcatgccatttggagcttcttcctgtttggatcactagaaggaggaggtcactcattacagttctcatatacagtcgttggttggttggttggttggttggttggtagattgattgattgattgattgattgattgattgattgattgattgattgattgattgattgattgattgattgattgattgattgattgattgattgattgattggtagtcaaaataagaaataatttccacagattcattacagaaatgattaaatgcatacataaaaaactggggggggggggatacaacaacacacttaagtcacatttgcctacgtaaagaaaagtaaagaaaatcaatagctatattttacatctcctttttttgctgtcttttaattagccttgttttgctgttatcttgattgaaactgtaacttcttcacctgcttcttttctttgtaggttttgccagcccagaaacaggcatggctgtgcaaggccagagcaccatgcacaatgcgctgcatgtcttcatgaacggctcaatgtcctcagtccagggctcagccaacgaccccatcttcctccttcaccatgctttcattgacaggtaacaaacacgtcatgacattagactgcacagtttttgacaaagttcatacaatctgttgtttatagctgctacaattagtgaagtttgtgaatgtacttggatgagcagcgaaagatcaattgagatcaattgttagagtttggttgccctgcagagcaaagaacaaaaaataatctggtggctttactgcgtgaggttattattggtggaatagaaacacaaaacataattgcatttatttgtttaattttttatcttatcttaactttcatcttgcatatttgtttcttacatcatttctagcatctttgagcgctggctaagaactcatcagcctccccggtccatctacccacgtaccaatgcaccaattggccacaatgacggctactacatggtgccattccttcctctttataggaatggagactacctcctgtccaacaaggctcttggatacgagtacgcctacctgttggacccaggtcattgcacaacaccagaaatgccctctgatctgcaaaagacgtgaatatctgttcagacacccatatccactctgttccacacaggtcagaggtttgtccaggagttcttgacagaggtgtaaaaagtactcaaaaattttactcaagtgaaagtacaagtacttagggaaaattttactcaattaaaagtaaaagtatctggctagaatcttacttgagtaaaagtaaaaaagtactccattaaaattgtacttgagtattaaggaagtaaaagtaaaagcaagaaagaaaactagagattcttgtttaagcttttaatctcaaaaaacattaaatgaaatgcatacaaggttttatcctgctttagaactgtttgtatttaattatcaaactataagacagacaatctaatgccagtacacgctactcaaagttgtaaaacctcagatttaacttcagtagaagctgattctcaaaattgttagtgtcaagcctagctcttttggggctgaaaagcaatcctgcagtgctgaaaagcctctcacaggcagccgatgcgggaagaggtgtattagtcttgatagagaggctgcaaatagcaggaaacgtgagcagagactccctggtgtctgaaacacaggccagatgggccctcgagcaggaaacagctatgaccatgattacgccaagctatcaactttgtatagaaaagttggtaatacgactcactatagggcgaattgggtaccgggccccccctcgaggtcgacggtatcgataagcttaggcctccaaggcggagtactgtcctccgggctggcggagtactgtcctccggcaaggtcggagtactgtcctccgacactagaggtcggagtactgtcctccgacgcaaggcggagtactgtcctccgggctggcggagtactgtcctccggcaaggtcggagtactgtcctccgacactagaggtcggagtactgtcctccgacgcaaggcggagtactgtcctccgggctggcggagtactgtcctccggcaagggtcgactctagagggtatataatggatcccatcgcgtctcagcctcactttgagctcctccacacgaattcctgcagcccgggggatccactagttctagagcggccgccaccgcggtggagctccagcttttgttccctttagtgagggttaattcaagtttgtacaaaaaagcaggctatggtgagcaagggcgaggagctgttcaccggggtggtgcccatcctggtcgagctggacggcgacgtaaacggccacaagttcagcgtgtccggcgagggcgagggcgatgccacctacggcaagctgaccctgaagttcatctgcaccaccggcaagctgcccgtgccctggcccaccctcgtgaccaccctgacctacggcgtgcagtgcttcagccgctaccccgaccacatgaagcagcacgacttcttcaagtccgccatgcccgaaggctacgtccaggagcgcaccatcttcttcaaggacgacggcaactacaagacccgcgccgaggtgaagttcgagggcgacaccctggtgaaccgcatcgagctgaagggcatcgacttcaaggaggacggcaacatcctggggcacaagctggagtacaactacaacagccacaacgtctatatcatggccgacaagcagaagaacggcatcaaggtgaacttcaagatccgccacaacatcgaggacggcagcgtgcagctcgccgaccactaccagcagaacacccccatcggcgacggccccgtgctgctgcccgacaaccactacctgagcacccagtccgccctgagcaaagaccccaacgagaagcgcgatcacatggtcctgctggagttcgtgaccgccgccgggatcactctcggcatggacgagctgtacaagggaggcgctgcaggaggctctagaatgggaaaccaagagctagaggaggtgtttgttgctgttatccgaccaaaaaacacaaccagcctcaactccaaagaataccgtgctaaatcctatgagattttacttatcgaagttcccctggagggaaaagagaaaaagcggaagaaagtgctgcttgggactaaaattcacgccgacagtgaccggacaaagtcaattctggagtttgtggatgaaaccaccaagcccatatccaataaccagggcataatagggaagcgtgttgtgcacatgaggaagttcctgttagatggagacagtggaggaaaagaggcctcgttatttattgtgccaattaatgtcaaagacaacagcaagtccgtgcatcaccctgggagccccagtttctactgccttcaggacatcatgcgtgtgtgtagtgaaaccagtgctcatttctcctccagcacctcaaagatgctgctcgctctcgacaagtggttagcggagcagcacactgtgcctcacgctattcctgctctgttccggccggctccggtggaccgtgtgaaaactaacgtgagtaacccggcgtacgcagtggagaagcagacagacgggacgctgcacatgggctacacggctctggagatcaagagtaaactgatgtctctggagaaagcagatctgtgcatccagaacccgctgtacggctcagatctgcagtacaccaacagagtggacaaagtcatcatcaacccttactttggcttgggagctccagattactccaaaatccagattccaaagagagacaaatggcagcacagcatgaccagcgtcaccgaagacaaagagcgccagtgggtggatgatttccctctgcaccgaagcgcctgtgagggagacactgagcttttgtctaaattgctggatggcggattctcagtcaaacagctggacagcgaccattgggcacccattcattatgcatgctggcatgggaaggtggaggccactaaactgctgctggagaaaggcaactgtaaccccaacctgctgaacggccagctgagctctcctttacacttcgcagctatcggcggtcatgcagaaatcgtgcagctcctcctgcagcacccagagatcgacagacacatcgaggaccagcagaaacgatcgccgcttcaagtatgtgaagaaaacaagcagaacaactgggaggaaaccgtgaatctccttcaacaagccagcaataaaccatacgagaaggtgaggatttaccgtatggatggatcgtaccgctctgtggagctgaagcatgggaacaacaccaccgtgcagcagatcatggagggcatgagattatcacaggagacccagcagtattttaccatctggatctgctccgaaaaccttagtctgcagctgaagccgtaccacaagcccttgcagcacttacggatgtggagcgagatcgtgacggatctcactgctctggatccacagagagaaagtccacagctcttcctgcgcagagacgttcggctgcctttagaggtcgagaaaaaggttgaagatccgctgtccatcctcatcctatttgatgaagctcgtcactgcctccttaaaggtttcctctcgacgtcagataacaagctaatcacgctcgcaagcctcctcctgcagatcatctacggaaactacgacagcaagaagcacaaacagggctttctaaatgaggaaaacctgaaatccatagttcccatttcaaaggtcaagagcaaagcacatcactggactaacaggatacttcacgagtacaagagtctgagcactagtgagggtgtgagtaaagaaatgcatcacctccagaggctcttcctgcagaactgctgggatattcctacttatggtgcagcgtttttcacaggacaggtcttcactaaagccagctccagcacacacaaggtgatccgcgtgtatgtgggcgtcaacaccaaaggcctgcatctgatgaacatggagacaaaagtgcttcacctcagtctggagtatgggacatttatgtggcagctgggtcaggctgatcaatacgtgcaaatccacagtctggagaacaagaagaactttgtcgttcacaccaaacaggctggtcttatcgtgaagctgctgatgaagctgagtggacaaattgcaccaaacgacagagctgtgtctgataaatatgcgtatgggtaaacccagctttcttgtacaaagtggaattcactagtgatttaatagtgtgcattcagtgcaggatgttatgtatttattttctgtagtgcaaactttttcaaagaattttccagtctaagcttttcagtcaagaaaaaaaaaggcgtctgattatctgtgatattttaaataattagctcttaaatctggtgaaccaagtggccacaacacattaaatactgacgttctacagccatgtagcttcatctggtctggtttgttttggcaggcacttattttccggtgatagttggccacaagagtattgtctgagccattcagtgctagactgtcattctcaggtcagaatccaccccactgattctgctgacaacactgttcccaccatgagataatgccattccagagagatccatttgtaagcccctctttctgcagcacaggtatataaccagggctctgcctccactaaggccggcacacatcatttggggatctttgtactgtactagcctctattagcctcctacttgcgttcagttcacatcttttgttcatcaggtgcaataagttacagtaaggagttaccaggtctgacattaatcgaattccaccatggtgagcaagggcgaggagctgttcaccggggtggtgcccatcctggtcgagctggacggcgacgtaaacggccacaagttcagcgtgtccggcgagggcgagggcgatgccacctacggcaagctgaccctgaagttcatctgcaccaccggcaagctgcccgtgccctggcccaccctcgtgaccaccctgacctacggcgtgcagtgcttcagccgctaccccgaccacatgaagcagcacgacttcttcaagtccgccatgcccgaaggctacgtccaggagcgcaccatcttcttcaaggacgacggcaactacaagacccgcgccgaggtgaagttcgagggcgacaccctggtgaaccgcatcgagctgaagggcatcgacttcaaggaggacggcaacatcctggggcacaagctggagtacaactacaacagccacaacgtctatatcatggccgacaagcagaagaacggcatcaaggtgaacttcaagatccgccacaacatcgaggacggcagcgtgcagctcgccgaccactaccagcagaacacccccatcggcgacggccccgtgctgctgcccgacaaccactacctgagcacccagtccgccctgagcaaagaccccaacgagaagcgcgatcacatggtcctgctggagttcgtgaccgccgccgggatcactctcggcatggacgagctgtacaagggcggtggaagatctgggaattcaaggcctctcgagcctctagattctgcagccctatagtgagtcgtattacgtagatccagacatgataagatacattgatgagtttggacaaaccacaactagaatgcagtgaaaaaaatgctttatttgtgaaatttgtgatgctattgctttatttgtaaccattataagctgcaataaacaagttaacaacaacaattgcattcattttatgtttcaggttcagggggaggtgtgggaggttttttccaactttattatacatagttgataattcactggccgtcgttttacatcgatgatgatccagacatgataagatacattgatgagtttggacaaaccacaactagaatgcagtgaaaaaaatgctttatttgtgaaatttgtgatgctattgctttatttgtaaccattataagctgcaataaacaagttaacaacaacaattgcattcattttatgtttcaggttcagggggaggtgtgggaggttttttaaagcaagtaaaacctctacaaatgtggtatggctgattatgatcctctagatcagatctgcgaagatacggccacgggtgctcttgatcctgtggctgattttggactgtgctgctcgcagctgctgatgaatcacatacttcctccattttcttccactgattgactgttataatttccctaatttccaggtcaaggtgctgtgcattgtggtaatagatgtgacatgacgtcacttccaaaggaccaatgaacatgtctgaccaatttcatataatgtgaaaacgattttcataggcagaataaataacatttaaattaaactgggcatcagcgcaattcaattggtttggtaatagcaagggaaaatagaatgaagtgatctccaaaaaataagtactttttgactgtaaataaaattgtaaggagtaaaaagtacttttttttctaaaaaaatgtaattaagtaaaagtaaaagtattgatttttaattgtactcaagtaaagtaaaaatccccaaaaataatacttaagtacagtaatcaagtaaaattactcaagtactttacacctctggttcttgaccccctaccttcagcaagcccagcagatccactagttctagagcggccgccaccgcggtggagctccagcttttgttccctttagtgagggttaattgcgcgcttggcgtaatcatggtcatagctgtttcctgtgtgaaattgttatccgctcacaattccacacaacatacgagccggaagcataaagtgtaaagcctggggtgcctaatgagtgagctaactcacattaattgcgttgcgctcactgcccgctttccagtcgggaaacctgtcgtgccagctgcattaatgaatcggccaacgcgcggggagaggcggtttgcgtattgggcgctcttccgcttcctcgctcactgactcgctgcgctcggtcgttcggctgcggcgagcggtatcagctcactcaaaggcggtaatacggttatccacagaatcaggggataacgcaggaaagaacatgtgagcaaaaggccagcaaaaggccaggaaccgtaaaaaggccgcgttgctggcgtttttccataggctccgcccccctgacgagcatcacaaaaatcgacgctcaagtcagaggtggcgaaacccgacaggactataaagataccaggcgtttccccctggaagctccctcgtgcgctctcctgttccgaccctgccgcttaccggatacctgtccgcctttctcccttcgggaagcgtggcgctttctcatagctcacgctgtaggtatctcagttcggtgtaggtcgttcgctccaagctgggctgtgtgcacgaaccccccgttcagcccgaccgctgcgccttatccggtaactatcgtcttgagtccaacccggtaagacacgacttatcgccactggcagcagccactggtaacaggattagcagagcgaggtatgtaggcggtgctacagagttcttgaagtggtggcctaactacggctacactagaaggacagtatttggtatctgcgctctgctgaagccagttaccttcggaaaaagagttggtagctcttgatccggcaaacaaaccaccgctggtagcggtggtttttttgtttgcaagcagcagattacgcgcagaaaaaaaggatctcaagaagatcctttgatcttttctacggggtctgacgctcagtggaacgaaaactcacgttaagggattttggtcatgagattatcaaaaaggatcttcacctagatccttttaaattaaaaatgaagttttaaatcaatctaaagtatatatgagtaaacttggtctgacagttaccaatgcttaatcagtgaggcacctatctcagcgatctgtctatttcgttcatccatagttgcctgactccccgtcgtgtagataactacgatacgggagggcttaccatctggccccagtgctgcaatgataccgcgagacccacgctcaccggctccagatttatcagcaataaaccagccagccggaagggccgagcgcagaagtggtcctgcaactttatccgcctccatccagtctattaattgttgccgggaagctagagtaagtagttcgccagttaatagtttgcgcaacgttgttgccattgctacaggcatcgtggtgtcacgctcgtcgtttggtatggcttcattcagctccggttcccaacgatcaaggcgagttacatgatcccccatgttgtgcaaaaaagcggttagctccttcggtcctccgatcgttgtcagaagtaagttggccgcagtgttatcactcatggttatggcagcactgcataattctcttactgtcatgccatccgtaagatgcttttctgtgactggtgagtactcaaccaagtcattctgagaatagtgtatgcggcgaccgagttgctcttgcccggcgtcaatacgggataataccgcgccacatagcagaactttaaaagtgctcatcattggaaaacgttcttcggggcgaaaactctcaaggatcttaccgctgttgagatccagttcgatgtaacccactcgtgcacccaactgatcttcagcatcttttactttcaccagcgtttctgggtgagcaaaaacaggaaggcaaaatgccgcaaaaaagggaataagggcgacacggaaatgttgaatactcatactcttcctttttcaatattattgaagcatttatcagggttattgtctcatgagcggatacatatttgaatgtatttagaaaaataaacaaataggggttccgcgcacatttccccgaaaagtg

SEQ ID NO: 13 - DNA, 484 bp, Artificial Sequence
  UAS promoter sequence
gtaatacgactcactatagggcgaattgggtaccgggccccccctcgaggtcgacggtatcgataagcttaggcctccaaggcggagtactgtcctccgggctggcggagtactgtcctccggcaaggtcggagtactgtcctccgacactagaggtcggagtactgtcctccgacgcaaggcggagtactgtcctccgggctggcggagtactgtcctccggcaaggtcggagtactgtcctccgacactagaggtcggagtactgtcctccgacgcaaggcggagtactgtcctccgggctggcggagtactgtcctccggcaagggtcgactctagagggtatataatggatcccatcgcgtctcagcctcactttgagctcctccacacgaattcctgcagcccgggggatccactagttctagagcggccgccaccgcggtggagctccagcttttgttccctttagtgagggttaatt

SEQ ID NO: 14 - DNA, 2955 bp, Artificial Sequence
  Coding nucleotide sequence of an mCherry-KRIT1 fusion protein including a linker sequence
atggtgagcaagggcgaggacgacaacatggccatcatcaaggagttcatgcgcttcaaggtgcacatggagggctccgtgaacggccacgagttcgagatcgagggcgagggcgagggccgcccctacgagggcacccagaccgccaagctgaaggtgaccaagggcggccccctgcccttcgcctgggacatcctgtcccctcagttcatgtacggctccaaggcctacgtgaagcaccccgccgacatccccgactacttgaagctgtccttccccgagggcttcaagtgggagcgcgtgatgaacttcgaggacggcggcgtggtgaccgtgacccaggactcctccctgcaggacggcgagttcatctacaaggtgaagctgcgcggcaccaacttcccctccgacggccccgtaatgcagaagaagaccatgggctgggaggcctcctccgagcggatgtaccccgaggacggcgccctgaagggcgagatcaagcagaggctgaagctgaaggacggcggccactacgacgccgaggtcaagaccacctacaaggccaagaagcccgtgcagctgcccggcgcctacaacgtcaacatcaagctggacatcacctcccacaacgaggactacaccatcgtggaacagtacgagcgcgccgagggccgccactccaccggcggcatggacgagctgtacaagggaggcgctgcaggaggctctagaatgggaaaccaagagctagaggaggtgtttgttgctgttatccgaccaaaaaacacaaccagcctcaactccaaagaataccgtgctaaatcctatgagattttacttatcgaagttcccctggagggaaaagagaaaaagcggaagaaagtgctgcttgggactaaaattcacgccgacagtgaccggacaaagtcaattctggagtttgtggatgaaaccaccaagcccatatccaataaccagggcataatagggaagcgtgttgtgcacatgaggaagttcctgttagatggagacagtggaggaaaagaggcctcgttatttattgtgccaattaatgtcaaagacaacagcaagtccgtgcatcaccctgggagccccagtttctactgccttcaggacatcatgcgtgtgtgtagtgaaaccagtgctcatttctcctccagcacctcaaagatgctgctcgctctcgacaagtggttagcggagcagcacactgtgcctcacgctattcctgctctgttccggccggctccggtggaccgtgtgaaaactaacgtgagtaacccggcgtacgcagtggagaagcagacagacgggacgctgcacatgggctacacggctctggagatcaagagtaaactgatgtctctggagaaagcagatctgtgcatccagaacccgctgtacggctcagatctgcagtacaccaacagagtggacaaagtcatcatcaacccttactttggcttgggagctccagattactccaaaatccagattccaaagagagacaaatggcagcacagcatgaccagcgtcaccgaagacaaagagcgccagtgggtggatgatttccctctgcaccgaagcgcctgtgagggagacactgagcttttgtctaaattgctggatggcggattctcagtcaaacagctggacagcgaccattgggcacccattcattatgcatgctggcatgggaaggtggaggccactaaactgctgctggagaaaggcaactgtaaccccaacctgctgaacggccagctgagctctcctttacacttcgcagctatcggcggtcatgcagaaatcgtgcagctcctcctgcagcacccagagatcgacagacacatcgaggaccagcagaaacgatcgccgcttcaagtatgtgaagaaaacaagcagaacaactgggaggaaaccgtgaatctccttcaacaagccagcaataaaccatacgagaaggtgaggatttaccgtatggatggatcgtaccgctctgtggagctgaagcatgggaacaacaccaccgtgcagcagatcatggagggcatgagattatcacaggagacccagcagtattttaccatctggatctgctccgaaaaccttagtctgcagctgaagccgtaccacaagcccttgcagcacttacggatgtggagcgagatcgtgacggatctcactgctctggatccacagagagaaagtccacagctcttcctgcgcagagacgttcggctgcctttagaggtcgagaaaaaggttgaagatccgctgtccatcctcatcctatttgatgaagctcgtcactgcctccttaaaggtttcctctcgacgtcagataacaagctaatcacgctcgcaagcctcctcctgcagatcatctacggaaactacgacagcaagaagcacaaacagggctttctaaatgaggaaaacctgaaatccatagttcccatttcaaaggtcaagagcaaagcacatcactggactaacaggatacttcacgagtacaagagtctgagcactagtgagggtgtgagtaaagaaatgcatcacctccagaggctcttcctgcagaactgctgggatattcctacttatggtgcagcgtttttcacaggacaggtcttcactaaagccagctccagcacacacaaggtgatccgcgtgtatgtgggcgtcaacaccaaaggcctgcatctgatgaacatggagacaaaagtgcttcacctcagtctggagtatgggacatttatgtggcagctgggtcaggctgatcaatacgtgcaaatccacagtctggagaacaagaagaactttgtcgttcacaccaaacaggctggtcttatcgtgaagctgctgatgaagctgagtggacaaattgcaccaaacgacagagctgtgtctgataaatatgcgtatgggtaa

SEQ ID NO: 15 - DNA, 708 bp, Artificial Sequence
  Coding nucleotide sequence of an mCherry
atggtgagcaagggcgaggacgacaacatggccatcatcaaggagttcatgcgcttcaaggtgcacatggagggctccgtgaacggccacgagttcgagatcgagggcgagggcgagggccgcccctacgagggcacccagaccgccaagctgaaggtgaccaagggcggccccctgcccttcgcctgggacatcctgtcccctcagttcatgtacggctccaaggcctacgtgaagcaccccgccgacatccccgactacttgaagctgtccttccccgagggcttcaagtgggagcgcgtgatgaacttcgaggacggcggcgtggtgaccgtgacccaggactcctccctgcaggacggcgagttcatctacaaggtgaagctgcgcggcaccaacttcccctccgacggccccgtaatgcagaagaagaccatgggctgggaggcctcctccgagcggatgtaccccgaggacggcgccctgaagggcgagatcaagcagaggctgaagctgaaggacggcggccactacgacgccgaggtcaagaccacctacaaggccaagaagcccgtgcagctgcccggcgcctacaacgtcaacatcaagctggacatcacctcccacaacgaggactacaccatcgtggaacagtacgagcgcgccgagggccgccactccaccggcggcatggacgagctgtacaag

SEQ ID NO: 16 - DNA, 24 bp, Artificial Sequence
  Coding nucleotide sequence of a linker that can be used for encoding a linker of a fusion protein of the invention.
ggaggcgctgcaggaggctctaga

SEQ ID NO: 17 - DNA, 586 bp, Artificial Sequence
  Nucleotide sequence of an alpha-crystallin promoter
aattcactagtgatttaatagtgtgcattcagtgcaggatgttatgtatttattttctgtagtgcaaactttttcaaagaattttccagtctaagcttttcagtcaagaaaaaaaaaggcgtctgattatctgtgatattttaaataattagctcttaaatctggtgaaccaagtggccacaacacattaaatactgacgttctacagccatgtagcttcatctggtctggtttgttttggcaggcacttattttccggtgatagttggccacaagagtattgtctgagccattcagtgctagactgtcattctcaggtcagaatccaccccactgattctgctgacaacactgttcccaccatgagataatgccattccagagagatccatttgtaagcccctctttctgcagcacaggtatataaccagggctctgcctccactaaggccggcacacatcatttggggatctttgtactgtactagcctctattagcctcctacttgcgttcagttcacatcttttgttcatcaggtgcaataagttacagtaaggagttaccaggtctgacattaatcgaatt

SEQ ID NO: 18 - DNA, 717 bp, Artificial Sequence
  Coding nucleotide sequence of an EGFP
atggtgagcaagggcgaggagctgttcaccggggtggtgcccatcctggtcgagctggacggcgacgtaaacggccacaagttcagcgtgtccggcgagggcgagggcgatgccacctacggcaagctgaccctgaagttcatctgcaccaccggcaagctgcccgtgccctggcccaccctcgtgaccaccctgacctacggcgtgcagtgcttcagccgctaccccgaccacatgaagcagcacgacttcttcaagtccgccatgcccgaaggctacgtccaggagcgcaccatcttcttcaaggacgacggcaactacaagacccgcgccgaggtgaagttcgagggcgacaccctggtgaaccgcatcgagctgaagggcatcgacttcaaggaggacggcaacatcctggggcacaagctggagtacaactacaacagccacaacgtctatatcatggccgacaagcagaagaacggcatcaaggtgaacttcaagatccgccacaacatcgaggacggcagcgtgcagctcgccgaccactaccagcagaacacccccatcggcgacggccccgtgctgctgcccgacaaccactacctgagcacccagtccgccctgagcaaagaccccaacgagaagcgcgatcacatggtcctgctggagttcgtgaccgccgccgggatcactctcggcatggacgagctgtacaag

SEQ ID NO: 19 - DNA, 2964 bp, Artificial Sequence
  Coding nucleotide sequence of an EGFP-KRIT1 fusion protein including a linker sequence
atggtgagcaagggcgaggagctgttcaccggggtggtgcccatcctggtcgagctggacggcgacgtaaacggccacaagttcagcgtgtccggcgagggcgagggcgatgccacctacggcaagctgaccctgaagttcatctgcaccaccggcaagctgcccgtgccctggcccaccctcgtgaccaccctgacctacggcgtgcagtgcttcagccgctaccccgaccacatgaagcagcacgacttcttcaagtccgccatgcccgaaggctacgtccaggagcgcaccatcttcttcaaggacgacggcaactacaagacccgcgccgaggtgaagttcgagggcgacaccctggtgaaccgcatcgagctgaagggcatcgacttcaaggaggacggcaacatcctggggcacaagctggagtacaactacaacagccacaacgtctatatcatggccgacaagcagaagaacggcatcaaggtgaacttcaagatccgccacaacatcgaggacggcagcgtgcagctcgccgaccactaccagcagaacacccccatcggcgacggccccgtgctgctgcccgacaaccactacctgagcacccagtccgccctgagcaaagaccccaacgagaagcgcgatcacatggtcctgctggagttcgtgaccgccgccgggatcactctcggcatggacgagctgtacaagggaggcgctgcaggaggctctagaatgggaaaccaagagctagaggaggtgtttgttgctgttatccgaccaaaaaacacaaccagcctcaactccaaagaataccgtgctaaatcctatgagattttacttatcgaagttcccctggagggaaaagagaaaaagcggaagaaagtgctgcttgggactaaaattcacgccgacagtgaccggacaaagtcaattctggagtttgtggatgaaaccaccaagcccatatccaataaccagggcataatagggaagcgtgttgtgcacatgaggaagttcctgttagatggagacagtggaggaaaagaggcctcgttatttattgtgccaattaatgtcaaagacaacagcaagtccgtgcatcaccctgggagccccagtttctactgccttcaggacatcatgcgtgtgtgtagtgaaaccagtgctcatttctcctccagcacctcaaagatgctgctcgctctcgacaagtggttagcggagcagcacactgtgcctcacgctattcctgctctgttccggccggctccggtggaccgtgtgaaaactaacgtgagtaacccggcgtacgcagtggagaagcagacagacgggacgctgcacatgggctacacggctctggagatcaagagtaaactgatgtctctggagaaagcagatctgtgcatccagaacccgctgtacggctcagatctgcagtacaccaacagagtggacaaagtcatcatcaacccttactttggcttgggagctccagattactccaaaatccagattccaaagagagacaaatggcagcacagcatgaccagcgtcaccgaagacaaagagcgccagtgggtggatgatttccctctgcaccgaagcgcctgtgagggagacactgagcttttgtctaaattgctggatggcggattctcagtcaaacagctggacagcgaccattgggcacccattcattatgcatgctggcatgggaaggtggaggccactaaactgctgctggagaaaggcaactgtaaccccaacctgctgaacggccagctgagctctcctttacacttcgcagctatcggcggtcatgcagaaatcgtgcagctcctcctgcagcacccagagatcgacagacacatcgaggaccagcagaaacgatcgccgcttcaagtatgtgaagaaaacaagcagaacaactgggaggaaaccgtgaatctccttcaacaagccagcaataaaccatacgagaaggtgaggatttaccgtatggatggatcgtaccgctctgtggagctgaagcatgggaacaacaccaccgtgcagcagatcatggagggcatgagattatcacaggagacccagcagtattttaccatctggatctgctccgaaaaccttagtctgcagctgaagccgtaccacaagcccttgcagcacttacggatgtggagcgagatcgtgacggatctcactgctctggatccacagagagaaagtccacagctcttcctgcgcagagacgttcggctgcctttagaggtcgagaaaaaggttgaagatccgctgtccatcctcatcctatttgatgaagctcgtcactgcctccttaaaggtttcctctcgacgtcagataacaagctaatcacgctcgcaagcctcctcctgcagatcatctacggaaactacgacagcaagaagcacaaacagggctttctaaatgaggaaaacctgaaatccatagttcccatttcaaaggtcaagagcaaagcacatcactggactaacaggatacttcacgagtacaagagtctgagcactagtgagggtgtgagtaaagaaatgcatcacctccagaggctcttcctgcagaactgctgggatattcctacttatggtgcagcgtttttcacaggacaggtcttcactaaagccagctccagcacacacaaggtgatccgcgtgtatgtgggcgtcaacaccaaaggcctgcatctgatgaacatggagacaaaagtgcttcacctcagtctggagtatgggacatttatgtggcagctgggtcaggctgatcaatacgtgcaaatccacagtctggagaacaagaagaactttgtcgttcacaccaaacaggctggtcttatcgtgaagctgctgatgaagctgagtggacaaattgcaccaaacgacagagctgtgtctgataaatatgcgtatgggtaa

SEQ ID NO: 20 - DNA, 25 bp, Artificial Sequence
  tnnt2a antisense sequence
catgtttgctctgatctgacacgca